European Patent Application EP 4 778 405 A1, published July 22, 2026. Title: 総合注意力、認知柔軟性及び／又は実行機能を改善するための組成物. Applicant: 江崎グリコ株式会社. The sequence listing filed with the application follows.

SEQUENCE LISTING (2 sequences)

SEQ ID NO: 1 - DNA, 22 bp, synthetic construct
  source 1..22: mol_type = other DNA
gattctggctcaggatgaacgc

SEQ ID NO: 2 - DNA, 20 bp, synthetic construct
  source 1..20: mol_type = other DNA
ctgataggacgcgaccccat